European Patent Application EP 4 455 157 A1, published October 30, 2024. Title: POLYNUCEOTIDE FOR T CELL SPECIFIC TRANSGENE EXPRESSION. Applicant: FUNDACION PUBLICA ANDALUZA PROGRESO Y SALUD- FPS. The sequence listing filed with the application follows.

SEQUENCE LISTING (8 sequences)

SEQ ID NO: 1 - DNA, 322 bp, synthetic construct
  source 1..322: mol_type = other DNA
ttagggttcaggcctgagcccctgctgctatccctccttcaaaggaggagatcaaggagcttagggtcccccgcacaggcccaccccagggtggggttcttcctttgaagggaattgctttggggtggggtcggttctatctgctccactctgtggctgacagtttctccaaggggctgcaggtgtcagctgtctgagcccgggctgagctctgaaacgtgcctactcaaacttcccgtggggtaggggaggcccagaaccaccctctgagagtggcaaaaagtggtcctggagccaggggaaatgtggatggggtagagat

SEQ ID NO: 2 - DNA, 116 bp, synthetic construct
  source 1..116: mol_type = other DNA
cttatcaaaattgagtcacttggacacatccagctgtgagggaggcctcaacttcctggaagttgggttttattttgcttgggcaagttggccatatgcccccaactgcctattta

SEQ ID NO: 3 - DNA, 190 bp, synthetic construct
  source 1..190: mol_type = other DNA
agcctgattctgcttaactttttcccttgactttggcattttcactttgacatgttccctgagagcctggggggtggggaacccagctccagctggtgacgtttggggccggcccaggcctagggtgtggaggagccttgccatcgggcttcctgtctctcttcatttaagcacgactctgcagaaggaa

SEQ ID NO: 4 - DNA, 79 bp, synthetic construct
  source 1..79: mol_type = other DNA
caaagcaccctccccactgggctcctggttgcagagctccaagtcctcacacagatacgcctgtttgagaagcagcggg

SEQ ID NO: 5 - DNA, 135 bp, synthetic construct
  source 1..135: mol_type = other DNA
caaagacgcaagcccagaggtaaggtggtcagactcggcttccttccccggagctgagagggaggggaacgtggggcagatgcacaggaagaatttctgtgctctgcccagttgtctgctttagataaatatgtc

SEQ ID NO: 6 - DNA, 187 bp, synthetic construct
  source 1..187: mol_type = other DNA
tgggggttatggggagaagataaaagtgcctgtgggaccacagactctcgctgtggtggagctgggccctcttaccctcccaagcctcgcccctcatcccatccctgggggccaggggtgagggcggcaggaacctcaaggctctgagaaagtgcgtggtgtgtgttgccattttggtctcttctcc

SEQ ID NO: 7 - DNA, 1029 bp, synthetic construct
  source 1..1029: mol_type = other DNA
ttagggttcaggcctgagcccctgctgctatccctccttcaaaggaggagatcaaggagcttagggtcccccgcacaggcccaccccagggtggggttcttcctttgaagggaattgctttggggtggggtcggttctatctgctccactctgtggctgacagtttctccaaggggctgcaggtgtcagctgtctgagcccgggctgagctctgaaacgtgcctactcaaacttcccgtggggtaggggaggcccagaaccaccctctgagagtggcaaaaagtggtcctggagccaggggaaatgtggatggggtagagatcttatcaaaattgagtcacttggacacatccagctgtgagggaggcctcaacttcctggaagttgggttttattttgcttgggcaagttggccatatgcccccaactgcctatttaagcctgattctgcttaactttttcccttgactttggcattttcactttgacatgttccctgagagcctggggggtggggaacccagctccagctggtgacgtttggggccggcccaggcctagggtgtggaggagccttgccatcgggcttcctgtctctcttcatttaagcacgactctgcagaaggaacaaagcaccctccccactgggctcctggttgcagagctccaagtcctcacacagatacgcctgtttgagaagcagcgggcaaagacgcaagcccagaggtaaggtggtcagactcggcttccttccccggagctgagagggaggggaacgtggggcagatgcacaggaagaatttctgtgctctgcccagttgtctgctttagataaatatgtctgggggttatggggagaagataaaagtgcctgtgggaccacagactctcgctgtggtggagctgggccctcttaccctcccaagcctcgcccctcatcccatccctgggggccaggggtgagggcggcaggaacctcaaggctctgagaaagtgcgtggtgtgtgttgccattttggtctcttctcc

SEQ ID NO: 8 - DNA, 1085 bp, synthetic construct
  source 1..1085: mol_type = other DNA
ttgaattcggcatgcttatcgattttagggttcaggcctgagcccctgctgctatccctccttcaaaggaggagatcaaggagcttagggtcccccgcacaggcccaccccagggtggggttcttcctttgaagggaattgctttggggtggggtcggttctatctgctccactctgtggctgacagtttctccaaggggctgcaggtgtcagctgtctgagcccgggctgagctctgaaacgtgcctactcaaacttcccgtggggtaggggaggcccagaaccaccctctgagagtggcaaaaagtggtcctggagccaggggaaatgtggatggggtagagatcttatcaaaattgagtcacttggacacatccagctgtgagggaggcctcaacttcctggaagttgggttttattttgcttgggcaagttggccatatgcccccaactgcctatttaagcctgattctgcttaactttttcccttgactttggcattttcactttgacatgttccctgagagcctggggggtggggaacccagctccagctggtgacgtttggggccggcccaggcctagggtgtggaggagccttgccatcgggcttcctgtctctcttcatttaagcacgactctgcagaaggaacaaagcaccctccccactgggctcctggttgcagagctccaagtcctcacacagatacgcctgtttgagaagcagcgggcaaagacgcaagcccagaggtaaggtggtcagactcggcttccttccccggagctgagagggaggggaacgtggggcagatgcacaggaagaatttctgtgctctgcccagttgtctgctttagataaatatgtctgggggttatggggagaagataaaagtgcctgtgggaccacagactctcgctgtggtggagctgggccctcttaccctcccaagcctcgcccctcatcccatccctgggggccaggggtgagggcggcaggaacctcaaggctctgagaaagtgcgtggtgtgtgttgccattttggtctcttctccggcgcgcccgggatccacgcgtctgaattcga